European Patent Specification EP 2 847 333 B1, published July 30, 2025. Title: BI-FUNCTIONAL SHORT-HAIRPIN RNA (BI-SHRNA) SPECIFIC FOR SINGLE-NUCLEOTIDE KRAS MUTATIONS. Applicant: STRIKE BIO, INC. Application EP 13788485.4. The sequence listing filed with the application follows.

SEQUENCE LISTING (58 sequences)

SEQ ID NO: 1 - DNA, 245 bp, Homo sapiens
tcgactgctgttgaagtgagcgcctgtggtagttggagctgattagtgaagccacagatgtaatcagctccaactaccacagttgcctactgcctcggaagcagctcactacattactcagctgttgaagtgagcgcctgtggtaggaagagatgattagtgaagccacagatgtaatcagctccaactaccacagttgcctactgcctcggaagcttaataaaggatcttttattttcattggc

SEQ ID NO: 2 - DNA, 245 bp, Homo sapiens
tcgactgctgttgaagtgagcgccgtggtagttggagctgatgtagtgaagccacagatgtacatcagctccaactaccacgttgcctactgcctcggaagcagctcactacattactcagctgttgaagtgagcgccgtggtagtcttagctaatgtagtgaagccacagatgtacatcagctccaactaccacgttgcctactgcctcggaagcttaataaaggatcttttattttcattggc

SEQ ID NO: 3 - DNA, 245 bp, Homo sapiens
tcgactgctgttgaagtgagcgcctggtagttggagctgatggtagtgaagccacagatgtaccatcagctccaactaccagttgcctactgcctcggaagcagctcactacattactcagctgttgaagtgagcgcctggtagttactgctaatggtagtgaagccacagatgtaccatcagctccaactaccagttgcctactgcctcggaagcttaataaaggatcttttattttcattggc

SEQ ID NO: 4 - DNA, 245 bp, Homo sapiens
tcgactgctgttgaagtgagcgccggtagttggagctgatggctagtgaagccacagatgtagccatcagctccaactaccgttgcctactgcctcggaagcagctcactacattactcagctgttgaagtgagcgccggtagttgtctctgatagctagtgaagccacagatgtagccatcagctccaactaccgttgcctactgcctcggaagcttaataaaggatcttttattttcattggc

SEQ ID NO: 5 - DNA, 245 bp, Homo sapiens
tcgactgctgttgaagtgagcgccgtagttggagctgatggcgtagtgaagccacagatgtacgccatcagctccaactacgttgcctactgcctcggaagcagctcactacattactcagctgttgaagtgagcgccgtagttggagctgatggcgtagtgaagccacagatgtacgccatcagctccaactacgttgcctactgcctcggaagcttaataaaggatcttttattttcattggc

SEQ ID NO: 6 - DNA, 245 bp, Homo sapiens
tcgactgctgttgaagtgagcgcctagttggagctgatggcgttagtgaagccacagatgtaacgccatcagctccaactagttgcctactgcctcggaagcagctcactacattactcagctgttgaagtgagcgcctagttggatgagatgacgttagtgaagccacagatgtaacgccatcagctccaactagttgcctactgcctcggaagcttaataaaggatcttttattttcattggc

SEQ ID NO: 7 - DNA, 245 bp, Homo sapiens
tcgactgctgttgaagtgagcgccagttggagctgatggcgtatagtgaagccacagatgtatacgccatcagctccaactgttgcctactgcctcggaagcagctcactacattactcagctgttgaagtgagcgccagttggagactatggagtatagtgaagccacagatgtatacgccatcagctccaactgttgcctactgcctcggaagcttaataaaggatcttttattttcattggc

SEQ ID NO: 8 - DNA, 245 bp, Homo sapiens
tcgactgctgttgaagtgagcgccgttggagctgatggcgtagtagtgaagccacagatgtactacgccatcagctccaacgttgcctactgcctcggaagcagctcactacattactcagctgttgaagtgagcgccgttgaagcacgtggtgtagtagtgaagccacagatgtactacgccatcagctccaacgttgcctactgcctcggaagcttaataaaggatcttttattttcattggc

SEQ ID NO: 9 - DNA, 245 bp, Homo sapiens
tcgactgctgttgaagtgagcgccttggagctgatggcgtaggtagtgaagccacagatgtacctacgccatcagctccaagttgcctactgcctcggaagcagctcactacattactcagctgttgaagtgagcgccttggagctataggtctaggtagtgaagccacagatgtacctacgccatcagctccaagttgcctactgcctcggaagcttaataaaggatcttttattttcattggc

SEQ ID NO: 10 - DNA, 245 bp, Homo sapiens
tcgactgctgttgaagtgagcgcctggagctgatggcgtaggctagtgaagccacagatgtagcctacgccatcagctccagttgcctactgcctcggaagcagctcactacattactcagctgttgaagtgagcgcctggagctgtatgcgttcgctagtgaagccacagatgtagcctacgccatcagctccagttgcctactgcctcggaagcttaataaaggatcttttattttcattggc

SEQ ID NO: 11 - DNA, 245 bp, Homo sapiens
tcgactgctgttgaagtgagcgccgttggagctgatggcgtagtagtgaagccacagatgtactatgccatcagctccaacgttgcctactgcctcggaagcagctcactacattactcagctgttgaagtgagcgccgttgaagcacgtggtgtagtagtgaagccacagatgtactatgccatcagctccaacgttgcctactgcctcggaagcttaataaaggatcttttattttcattggc

SEQ ID NO: 12 - DNA, 245 bp, Homo sapiens
tcgactgctgttgaagtgagcgccttggagctgatggcgtaggtagtgaagccacagatgtacctatgccatcagctccaagttgcctactgcctcggaagcagctcactacattactcagctgttgaagtgagcgccttggagctataggtctaggtagtgaagccacagatgtacctatgccatcagctccaagttgcctactgcctcggaagcttaataaaggatcttttattttcattggc

SEQ ID NO: 13 - DNA, 245 bp, Homo sapiens
tcgactgctgttgaagtgagcgcctggagctgatggcgtaggctagtgaagccacagatgtagcctatgccatcagctccagttgcctactgcctcggaagcagctcactacattactcagctgttgaagtgagcgcctggagctgtatgcgttcgctagtgaagccacagatgtagcctatgccatcagctccagttgcctactgcctcggaagcttaataaaggatcttttattttcattggc

SEQ ID NO: 14 - DNA, 245 bp, Homo sapiens
tcgactgctgttgaagtgagcgccgttggagctcatggcgtagtagtgaagccacagatgtactacgccatgagctccaacgttgcctactgcctcggaagcagctcactacattactcagctgttgaagtgagcgccgttgaagcacgtggtgtagtagtgaagccacagatgtactacgccatgagctccaacgttgcctactgcctcggaagcttaataaaggatcttttattttcattggc

SEQ ID NO: 15 - DNA, 245 bp, Homo sapiens
tcgactgctgttgaagtgagcgccttggagctcatggcgtaggtagtgaagccacagatgtacctacgccatgagctccaagttgcctactgcctcggaagcagctcactacattactcagctgttgaagtgagcgccttggagctataggtctaggtagtgaagccacagatgtacctacgccatgagctccaagttgcctactgcctcggaagcttaataaaggatcttttattttcattggc

SEQ ID NO: 16 - DNA, 245 bp, Homo sapiens
tcgactgctgttgaagtgagcgcctggagctcatggcgtaggctagtgaagccacagatgtagcctacgccatgagctccagttgcctactgcctcggaagcagctcactacattactcagctgttgaagtgagcgcctggagctgtatgcgttcgctagtgaagccacagatgtagcctacgccatgagctccagttgcctactgcctcggaagcttaataaaggatcttttattttcattggc

SEQ ID NO: 17 - DNA, 245 bp, Homo sapiens
tcgactgctgttgaagtgagcgccgtggtagttggagctgttgtagtgaagccacagatgtacaacagctccaactaccacgttgcctactgcctcggaagcagctcactacattactcagctgttgaagtgagcgccgtggtagtcttagctattgtagtgaagccacagatgtacaacagctccaactaccacgttgcctactgcctcggaagcttaataaaggatcttttattttcattggc

SEQ ID NO: 18 - DNA, 245 bp, Homo sapiens
tcgactgctgttgaagtgagcgcctggtagttggagctgttggtagtgaagccacagatgtaccaacagctccaactaccagttgcctactgcctcggaagcagctcactacattactcagctgttgaagtgagcgcctggtagttactgctattggtagtgaagccacagatgtaccaacagctccaactaccagttgcctactgcctcggaagcttaataaaggatcttttattttcattggc

SEQ ID NO: 19 - DNA, 245 bp, Homo sapiens
tcgactgctgttgaagtgagcgcctgtggtagttggagctcgttagtgaagccacagatgtaacgagctccaactaccacagttgcctactgcctcggaagcagctcactacattactcagctgttgaagtgagcgcctgtggtagactgagctagttagtgaagccacagatgtaacgagctccaactaccacagttgcctactgcctcggaagcttaataaaggatcttttattttcattggc

SEQ ID NO: 20 - DNA, 245 bp, Homo sapiens
tcgactgctgttgaagtgagcgccgtggtagttggagctcgtgtagtgaagccacagatgtacacgagctccaactaccacgttgcctactgcctcggaagcagctcactacattactcagctgttgaagtgagcgccgtggtagtactagctagtgtagtgaagccacagatgtacacgagctccaactaccacgttgcctactgcctcggaagcttaataaaggatcttttattttcattggc

SEQ ID NO: 21 - DNA, 245 bp, Homo sapiens
tcgactgctgttgaagtgagcgcctgtggtagttggagcttgttagtgaagccacagatgtaacaagctccaactaccacagttgcctactgcctcggaagcagctcactacattactcagctgttgaagtgagcgcctgtggtagactgagctagttagtgaagccacagatgtaacaagctccaactaccacagttgcctactgcctcggaagcttaataaaggatcttttattttcattggc

SEQ ID NO: 22 - DNA, 245 bp, Homo sapiens
tcgactgctgttgaagtgagcgccgtggtagttggagcttgtgtagtgaagccacagatgtacacaagctccaactaccacgttgcctactgcctcggaagcagctcactacattactcagctgttgaagtgagcgccgtggtagtcttagcttatgtagtgaagccacagatgtacacaagctccaactaccacgttgcctactgcctcggaagcttaataaaggatcttttattttcattggc

SEQ ID NO: 23 - DNA, 208 bp, Homo sapiens
gctagccaccatgactgaatataaacttgtggtagttggagctggtggcgtaggcaagagtgcttccaaggtgtacgaccccgagcaacgcaaacgcatgatcactgggcctcagtggtgggctcgctgcaagcaaatgaacgtgctggactccttcatcaactactatgattccgagaagcacgccgaggaggcacgtcgtgcctca

SEQ ID NO: 24 - DNA, 51 bp, Homo sapiens
atgactgaatataaacttgtggtagttggagctgatggcgtaggcaagagt

SEQ ID NO: 25 - DNA, 208 bp, Homo sapiens
cacttcgcatattaaggtgacgcgtgtggcctcgaacaccgagcgaccctgcagcgacccgcttaaaagcttggcattccggtactgttggtaaagccaccatgactgaatataaacttgtggtagttggagctgatggcgtaggcaagagtgccgatgctaagaacattaagaagggccctgctcccttctaccctctggaggatgg

SEQ ID NO: 26 - DNA, 36 bp, Homo sapiens
cttgtggtagttggagctggtggcgtaggcaagagt

SEQ ID NO: 27 - DNA, 30 bp, Homo sapiens
cttgtggtagttggagctgatggcgtaggc

SEQ ID NO: 28 - DNA, 30 bp, Homo sapiens
cttgtggtagttggagctgttggcgtaggc

SEQ ID NO: 29 - DNA, 30 bp, Homo sapiens
cttgtggtagttggagctcgtggcgtaggc

SEQ ID NO: 30 - DNA, 30 bp, Homo sapiens
cttgtggtagttggagcttgtggcgtaggc

SEQ ID NO: 31 - DNA, 19 bp, Homo sapiens
atcagctccaactaccaca

SEQ ID NO: 32 - DNA, 19 bp, Homo sapiens
catcagctccaactaccac

SEQ ID NO: 33 - DNA, 19 bp, Homo sapiens
ccatcagctccaactacca

SEQ ID NO: 34 - DNA, 19 bp, Homo sapiens
gccatcagctccaactacc

SEQ ID NO: 35 - DNA, 19 bp, Homo sapiens
cgccatcagctccaactac

SEQ ID NO: 36 - DNA, 19 bp, Homo sapiens
acgccatcagctccaacta

SEQ ID NO: 37 - DNA, 19 bp, Homo sapiens
tacgccatcagctccaact

SEQ ID NO: 38 - DNA, 19 bp, Homo sapiens
ctacgccatcagctccaac

SEQ ID NO: 39 - DNA, 19 bp, Homo sapiens
cctacgccatcagctccaa

SEQ ID NO: 40 - DNA, 19 bp, Homo sapiens
gcctacgccatcagctcca

SEQ ID NO: 41 - DNA, 19 bp, Homo sapiens
ctatgccatcagctccaac

SEQ ID NO: 42 - DNA, 19 bp, Homo sapiens
cctatgccatcagctccaa

SEQ ID NO: 43 - DNA, 19 bp, Homo sapiens
gcctatgccatcagctcca

SEQ ID NO: 44 - DNA, 19 bp, Homo sapiens
ctacgccatgagctccaac

SEQ ID NO: 45 - DNA, 19 bp, Homo sapiens
cctacgccatgagctccaa

SEQ ID NO: 46 - DNA, 19 bp, Homo sapiens
gcctacgccatgagctcca

SEQ ID NO: 47 - DNA, 19 bp, Homo sapiens
caacagctccaactaccac

SEQ ID NO: 48 - DNA, 19 bp, Homo sapiens
ccaacagctccaactacca

SEQ ID NO: 49 - DNA, 19 bp, Homo sapiens
acgagctccaactaccaca

SEQ ID NO: 50 - DNA, 19 bp, Homo sapiens
cacgagctccaactaccac

SEQ ID NO: 51 - DNA, 19 bp, Homo sapiens
acaagctccaactaccaca

SEQ ID NO: 52 - DNA, 19 bp, Homo sapiens
cacaagctccaactaccac

SEQ ID NO: 53 - DNA, 1280 bp, Homo sapiens
cgtcgtcgactttcttccccattagggattatgctgaatttgtatggtttatagttgttagagtttgaggtgttaattctaattatctatttcaaatttagcaggaaaaaagagaacatcaccttgtaaaactgaagattgtgaccatcgactgctgttgaagtgagcgccgtggtagttggagctgatgtagtgaagccacagatgtacatcagctccaactaccacgttgcctactgcctcggaagcagctgcctcgggaagccaagttgggctttaaagtgcagggcctgctgatgttgagtgcttttgctgttgaagtgagcgccgtggtagtcttagctaatgtagtgaagccacagatgtacatcagctccaactaccacgttgcctactgcctcggaagcttaataaaggatcttttattttcattggctaagaagttatgtattcatccaataattcaagccaagcaagtatataggtgttttaatagtttttgttttcgactgctgttgaagtgagcgcctggtagttggagctgttggtagtgaagccacagatgtaccaacagctccaactaccagttgcctactgcctcggaagctatttccttcaaatgaatgatttttactaattttgtgtacttttattgtgtcgatgtagaatctgcctggtctatctgatgtgacagcttctgctgttgaagtgagcgcctggtagttactgctattggtagtgaagccacagatgtaccaacagctccaactaccagttgcctactgcctcggaagcttaataaaggatcttttattttcattggctagctgtagaactccagcttcggcctgtcgcccaatcaaactgtcctgttactgaatcgactgctgttgaagtgagcgccgtggtagttggagctcgtgtagtgaagccacagatgtacacgagctccaactaccacgttgcctactgcctcggaagcaaaagtctgtagaaaagtaagggaaactcaaacccgctgttgaagtgagcgccgtggtagtactagctagtgtagtgaagccacagatgtacacgagctccaactaccacgttgcctactgcctcggaagcttaataaaggatcttttattttcattggctggggattgtgaccagaagattttgaaaattaaatattactgaagatttcgacttccactgttaaatgtacaagatacatgaaatattaaagaaaatgtgtaactttttgtgtaaatacatcttgtgcggccgcggat

SEQ ID NO: 54 - DNA, 1280 bp, Homo sapiens
cgtcgtcgactttcttccccattagggattatgctgaatttgtatggtttatagttgttagagtttgaggtgttaattctaattatctatttcaaatttagcaggaaaaaagagaacatcaccttgtaaaactgaagattgtgaccatcgactgctgttgaagtgagcgcctgtggtagttggagcttgttagtgaagccacagatgtaacaagctccaactaccacagttgcctactgcctcggaagcagctgcctcgggaagccaagttgggctttaaagtgcagggcctgctgatgttgagtgcttttgctgttgaagtgagcgcctgtggtagactgagctagttagtgaagccacagatgtaacaagctccaactaccacagttgcctactgcctcggaagcttaataaaggatcttttattttcattggctaagaagttatgtattcatccaataattcaagccaagcaagtatataggtgttttaatagtttttgttttcgactgctgttgaagtgagcgccgtggtagttggagctgatgtagtgaagccacagatgtacatcagctccaactaccacgttgcctactgcctcggaagctatttccttcaaatgaatgatttttactaattttgtgtacttttattgtgtcgatgtagaatctgcctggtctatctgatgtgacagcttctgctgttgaagtgagcgccgtggtagtcttagctaatgtagtgaagccacagatgtacatcagctccaactaccacgttgcctactgcctcggaagcttaataaaggatcttttattttcattggctagctgtagaactccagcttcggcctgtcgcccaatcaaactgtcctgttactgaatcgactgctgttgaagtgagcgcctggtagttggagctgttggtagtgaagccacagatgtaccaacagctccaactaccagttgcctactgcctcggaagcaaaagtctgtagaaaagtaagggaaactcaaacccgctgttgaagtgagcgcctggtagttactgctattggtagtgaagccacagatgtaccaacagctccaactaccagttgcctactgcctcggaagcttaataaaggatcttttattttcattggctggggattgtgaccagaagattttgaaaattaaatattactgaagatttcgacttccactgttaaatgtacaagatacatgaaatattaaagaaaatgtgtaactttttgtgtaaatacatcttgtgcggccgcggat

SEQ ID NO: 55 - DNA, 1029 bp, Homo sapiens
cgtcgtcgactttcttccccattagggattatgctgaatttgtatggtttatagttgttagagtttgaggtgttaattctaattatctatttcaaatttagcaggaaaaaagagaacatcaccttgtaaaactgaagattgtgaccagtcagaataatgtgtggtagttggagctgatgtgatatgtgcatctcatcagctccaactaccaccattatggtgacagctgcctcgggaagccaagttgggctttaaagtgcagggcctgctgatgttgagtgctttttgttcgtggtagtcttagctaatgtgaagtagattagcatctcatcagctccaactaccaccataagaagttatgtattcatccaataattcaagccaagcaagtatataggtgttttaatagtttttgtttgcagtcctctgtttggtagttggagctgttggagaagaatgtagtccaacagctccaactaccatggtggcctgctatttccttcaaatgaatgatttttactaattttgtgtacttttattgtgtcgatgtagaatctgcctggtctatctgatgtgacagcttctgtagcacttggtagttactgctattggtgtttagttatctccaacagctccaactaccatactgctagctgtagaactccagcttcggcctgtcgcccaatcaaactgtcctgttactgaacactgttctatggttgtggtagttggagctcgtgtgtgtgatattctgccacgagctccaactaccacctgtggtagtgaaaagtctgtagaaaagtaagggaaactcaaacccctttctacacgtggtagtactagctagtggtgtttctgtatggcacgagctccaactaccactgagtttggtggggattgtgaccagaagattttgaaaattaaatattactgaagatttcgacttccactgttaaatgtacaagatacatgaaatattaaagaaaatgtgtaactttttgtgtaaatacatcttgtgcggccgcggat

SEQ ID NO: 56 - DNA, 1029 bp, Homo sapiens
cgtcgtcgactttcttccccattagggattatgctgaatttgtatggtttatagttgttagagtttgaggtgttaattctaattatctatttcaaatttagcaggaaaaaagagaacatcaccttgtaaaactgaagattgtgaccagtcagaataatgttgtggtagttggagcttgttgatatgtgcatctacaagctccaactaccacacattatggtgacagctgcctcgggaagccaagttgggctttaaagtgcagggcctgctgatgttgagtgctttttgttctgtggtagactgagctagttgaagtagattagcatctacaagctccaactaccacacataagaagttatgtattcatccaataattcaagccaagcaagtatataggtgttttaatagtttttgtttgcagtcctctgttgtggtagttggagctgatgagaagaatgtagtcatcagctccaactaccactggtggcctgctatttccttcaaatgaatgatttttactaattttgtgtacttttattgtgtcgatgtagaatctgcctggtctatctgatgtgacagcttctgtagcactgtggtagtcttagctaatgtgtttagttatctcatcagctccaactaccactactgctagctgtagaactccagcttcggcctgtcgcccaatcaaactgtcctgttactgaacactgttctatggtttggtagttggagctgttggtgtgtgatattctgcccaacagctccaactaccactgtggtagtgaaaagtctgtagaaaagtaagggaaactcaaacccctttctacactggtagttactgctattgggtgtttctgtatggccaacagctccaactaccatgagtttggtggggattgtgaccagaagattttgaaaattaaatattactgaagatttcgacttccactgttaaatgtacaagatacatgaaatattaaagaaaatgtgtaactttttgtgtaaatacatcttgtgcggccgcggat

SEQ ID NO: 57 - DNA, 1050 bp, Homo sapiens
tttcttccccattagggattatgctgaatttgtatggtttatagttgttagagtttgaggtgttaattctaattatctatttcaaatttagcaggaaaaaagagaacatcaccttgtaaaactgaagattgtgaccagtcagaataatgtcaaagtgcttacagtgcaggtagtgatatgtgcatctactgcagtgaaggcacttgtagcattatggtgacagctgcctcgggaagccaagttgggctttaaagtgcagggcctgctgatgttgagtgctttttgttctaaggtgcatctagtgcagatagtgaagtagattagcatctactgccctaagtgctccttctggcataagaagttatgtattcatccaataattcaagccaagcaagtatataggtgttttaatagtttttgtttgcagtcctctgttagttttgcatagttgcactacaagaagaatgtagttgtgcaaatctatgcaaaactgatggtggcctgctatttccttcaaatgaatgatttttactaattttgtgtacttttattgtgtcgatgtagaatctgcctggtctatctgatgtgacagcttctgtagcactaaagtgcttatagtgcaggtagtgtttagttatctactgcattatgagcacttaaagtactgctagctgtagaactccagcttcggcctgtcgcccaatcaaactgtcctgttactgaacactgttctatggttagttttgcaggtttgcatccagctgtgtgatattctgctgtgcaaatccatgcaaaactgactgtggtagtgaaaagtctgtagaaaagtaagggaaactcaaacccctttctacacaggttgggatcggttgcaatgctgtgtttctgtatggtattgcacttgtcccggcctgttgagtttggtggggattgtgaccagaagattttgaaaattaaatattactgaagatttcgacttccactgttaaatgtacaagatacatgaaatattaaagaaaatgtgtaactttttgtgtaaatacatcttgt

SEQ ID NO: 58 - DNA, 51 bp, Homo sapiens
atgactgaatataaacttgtggtagttggagctggtggcgtaggcaagagt